European Patent Application EP 4 733 390 A2, published April 29, 2026. Title: LACTOBACILLUS PARACASEI STRAIN AND USE THEREOF. Applicant: Ko BioLabs, Inc. Application EP. The sequence listing filed with the application follows.

SEQUENCE LISTING (21 sequences)

SEQ ID NO: 1 - DNA, 1472 bp, Lactobacillus paracasei
  source 1..1472: mol_type = unassigned DNA
gcaggtggcgggtgctatacatgcagtcgacgagttctcgttgatgatcggtgcttgcaccgagattcaacatggaacgagtggcggacgggtgagtaacacgtgggtaacctgcccttaagtgggggataacatttggaaacagatgctaataccgcatagatccaagaaccgcatggttcttggctgaaagatggcgtaagctatcgcttttggatggacccgcggcgtattagctagttggtgaggtaatggctcaccaaggcgatgatacgtagccgaactgagaggttgatcggccacattgggactgagacacggcccaaactcctacgggaggcagcagtagggaatcttccacaatggacgcaagtctgatggagcaacgccgcgtgagtgaagaaggctttcgggtcgtaaaactctgttgttggagaagaatggtcggcagagtaactgttgtcggcgtgacggtatccaaccagaaagccacggctaactacgtgccagcagccgcggtaatacgtaggtggcaagcgttatccggatttattgggcgtaaagcgagcgcaggcggttttttaagtctgatgtgaaagccctcggcttaaccgaggaagcgcatcggaaactgggaaacttgagtgcagaagaggacagtggaactccatgtgtagcggtgaaatgcgtagatatatggaagaacaccagtggcgaaggcggctgtctggtctgtaactgacgctgaggctcgaaagcatgggtagcgaacaggattagataccctggtagtccatgccgtaaacgatgaatgctaggtgttggagggtttccgcccttcagtgccgcagctaacgcattaagcattccgcctggggagtacgaccgcaaggttgaaactcaaaggaattgacgggggcccgcacaagcggtggagcatgtggtttaattcgaagcaacgcgaagaaccttaccaggtcttgacatcttttgatcacctgagagatcaggtttccccttcgggggcaaaatgacaggtggtgcatggttgtcgtcagctcgtgtcgtgagatgttgggttaagtcccgcaacgagcgcaacccttatgactagttgccagcatttagttgggcactctagtaagactgccggtgacaaaccggaggaaggtggggatgacgtcaaatcatcatgccccttatgacctgggctacacacgtgctacaatggatggtacaacgagttgcgagaccgcgaggtcaagctaatctcttaaagccattctcagttcggactgtaggctgcaactcgcctacacgaagtcggaatcgctagtaatcgcggatcagcacgccgcggtgaatacgttcccgggccttgtacacaccgcccgtcacaccatgagagtttgtaacacccgaagccggtggcgtaaccctttagggagcgagcgtctaagtggctcacgcct

SEQ ID NO: 2 - DNA, 1479 bp, Lactobacillus paracasei
  source 1..1479: mol_type = unassigned DNA
gccagtggggggggtgctatacatgcagtcgaacgagttctcgttgatgatcggtgcttgcaccgagattcaacatggaacgagtggcggacgggtgagtaacacgtgggtaacctgcccttaagtgggggataacatttggaaacagatgctaataccgcatagatccaagaaccgcatggttcttggctgaaagatggcgtaagctatcgcttttggatggacccgcggcgtattagctagttggtgaggtaatggctcaccaaggcgatgatacgtagccgaactgagaggttgatcggccacattgggactgagacacggcccaaactcctacgggaggcagcagtagggaatcttccacaatggacgcaagtctgatggagcaacgccgcgtgagtgaagaaggctttcgggtcgtaaaactctgttgttggagaagaatggtcggcagagtaactgttgtcggcgtgacggtatccaaccagaaagccacggctaactacgtgccagcagccgcggtaatacgtaggtggcaagcgttatccggatttattgggcgtaaagcgagcgcaggcggttttttaagtctgatgtgaaagccctcggcttaaccgaggaagcgcatcggaaactgggaaacttgagtgcagaagaggacagtggaactccatgtgtagcggtgaaatgcgtagatatatggaagaacaccagtggcgaaggcggctgtctggtctgtaactgacgctgaggctcgaaagcatgggtagcgaacaggattagataccctggtagtccatgccgtaaacgatgaatgctaggtgttggagggtttccgcccttcagtgccgcagctaacgcattaagcattccgcctggggagtacgaccgcaaggttgaaactcaaaggaattgacgggggcccgcacaagcggtggagcatgtggtttaattcgaagcaacgcgaagaaccttaccaggtcttgacatcttttgatcacctgagagatcaggtttccccttcgggggcaaaatgacaggtggtgcatggttgtcgtcagctcgtgtcgtgagatgttgggttaagtcccgcaacgagcgcaacccttatgactagttgccagcatttagttgggcactctagtaagactgccggtgacaaaccggaggaaggtggggatgacgtcaaatcatcatgccccttatgacctgggctacacacgtgctacaatggatggtacaacgagttgcgagaccgcgaggtcaagctaatctcttaaagccattctcagttcggactgtaggctgcaactcgcctacacgaagtcggaatcgctagtaatcgcggatcagcacgccgcggtgaatacgttcccgggccttgtacacaccgcccgtcacaccatgagagtttgtaacacccgaagccggtggcgtaaccctttagggagcgagccgtctaaggtgaaccaaagtttg

SEQ ID NO: 3 - DNA, 1473 bp, Lactobacillus paracasei
  source 1..1473: mol_type = unassigned DNA
gcagttgggggggagctatacatgcagtcgacgagttctcgttgatgatcggtgcttgcaccgagattcaacatggaacgagtggcggacgggtgagtaacacgtgggtaacctgcccttaagtgggggataacatttggaaacagatgctaataccgcatagatccaagaaccgcatggttcttggctgaaagatggcgtaagctatcgcttttggatggacccgcggcgtattagctagttggtgaggtaatggctcaccaaggcgatgatacgtagccgaactgagaggttgatcggccacattgggactgagacacggcccaaactcctacgggaggcagcagtagggaatcttccacaatggacgcaagtctgatggagcaacgccgcgtgagtgaagaaggctttcgggtcgtaaaactctgttgttggagaagaatggtcggcagagtaactgttgccggcgtgacggtatccaaccagaaagccacggctaactacgtgccagcagccgcggtaatacgtaggtggcaagcgttatccggatttattgggcgtaaagcgagcgcaggcggttttttaagtctgatgtgaaagccctcggcttaaccgaggaagcgcatcggaaactgggaaacttgagtgcagaagaggacagtggaactccatgtgtagcggtgaaatgcgtagatatatggaagaacaccagtggcgaaggcggctgtctggtctgtaactgacgctgaggctcgaaagcatgggtagcgaacaggattagataccctggtagtccatgccgtaaacgatgaatgctaggtgttggagggtttccgcccttcagtgccgcagctaacgcattaagcattccgcctggggagtacgaccgcaaggttgaaactcaaaggaattgacgggggcccgcacaagcggtggagcatgtggtttaattcgaagcaacgcgaagaaccttaccaggtcttgacatcttttgatcacctgagagatcaggtttccccttcgggggcaaaatgacaggtggtgcatggttgtcgtcagctcgtgtcgtgagatgttgggttaagtcccgcaacgagcgcaacccttatgactagttgccagcatttagttgggcactctagtaagactgccggtgacaaaccggaggaaggtggggatgacgtcaaatcatcatgccccttatgacctgggctacacacgtgctacaatggatggtacaacgagttgcgagaccgcgaggtcaagctaatctcttaaagccattctcagttcggactgtaggctgcaactcgcctacacgaagtcggaatcgctagtaatcgcggatcagcacgccgcggtgaatacgttcccgggccttgtacacaccgcccgtcacaccatgagagtttgtaacacccgaagccggtggcgtaaccctttagggagcgagccgtctaagtgtacaaagtt

SEQ ID NO: 4 - DNA, 20 bp, synthetic construct
  misc_feature 1..20: note = primer
  source 1..20: mol_type = other DNA
ccagcagagaatggaaagtc

SEQ ID NO: 5 - DNA, 20 bp, synthetic construct
  misc_feature 1..20: note = primer
  source 1..20: mol_type = other DNA
gatgcttcttacatgtctcg

SEQ ID NO: 6 - DNA, 20 bp, synthetic construct
  misc_feature 1..20: note = primer
  source 1..20: mol_type = other DNA
ccccaaggaattgacagttg

SEQ ID NO: 7 - DNA, 21 bp, synthetic construct
  misc_feature 1..21: note = primer
  source 1..21: mol_type = other DNA
gggaaactaaagctcacaaac

SEQ ID NO: 8 - DNA, 19 bp, synthetic construct
  misc_feature 1..19: note = primer
  source 1..19: mol_type = other DNA
ctgcaatgcctgtgggctc

SEQ ID NO: 9 - DNA, 19 bp, synthetic construct
  misc_feature 1..19: note = primer
  source 1..19: mol_type = other DNA
gactgcagggactctcgct

SEQ ID NO: 10 - DNA, 20 bp, synthetic construct
  misc_feature 1..20: note = primer
  source 1..20: mol_type = other DNA
aagactcatcgccaaagcat

SEQ ID NO: 11 - DNA, 19 bp, synthetic construct
  misc_feature 1..19: note = primer
  source 1..19: mol_type = other DNA
tccacatgctggctacaca

SEQ ID NO: 12 - DNA, 17 bp, synthetic construct
  misc_feature 1..17: note = primer
  source 1..17: mol_type = other DNA
tcaagcactgccaggcg

SEQ ID NO: 13 - DNA, 18 bp, synthetic construct
  misc_feature 1..18: note = primer
  source 1..18: mol_type = other DNA
caggagcccttgtcggat

SEQ ID NO: 14 - DNA, 24 bp, synthetic construct
  misc_feature 1..24: note = primer
  source 1..24: mol_type = other DNA
acccgaaactgatgctgtggatag

SEQ ID NO: 15 - DNA, 24 bp, synthetic construct
  misc_feature 1..24: note = primer
  source 1..24: mol_type = other DNA
aaatggccgggcagaacttgtgta

SEQ ID NO: 16 - DNA, 20 bp, synthetic construct
  misc_feature 1..20: note = primer
  source 1..20: mol_type = other DNA
cagacgtccgtcagttttcg

SEQ ID NO: 17 - DNA, 20 bp, synthetic construct
  misc_feature 1..20: note = primer
  source 1..20: mol_type = other DNA
catggctgctggacttgaac

SEQ ID NO: 18 - DNA, 20 bp, synthetic construct
  misc_feature 1..20: note = primer
  source 1..20: mol_type = other DNA
gtctcccatcacggttcagt

SEQ ID NO: 19 - DNA, 20 bp, synthetic construct
  misc_feature 1..20: note = primer
  source 1..20: mol_type = other DNA
tgtcattccacactcccaga

SEQ ID NO: 20 - DNA, 21 bp, synthetic construct
  misc_feature 1..21: note = primer
  source 1..21: mol_type = other DNA
ttatggacaggactgaaagac

SEQ ID NO: 21 - DNA, 22 bp, synthetic construct
  misc_feature 1..22: note = primer
  source 1..22: mol_type = other DNA
gctttaatgtaatccagcaggt